European Patent Application EP 4 324 479 A2, published February 21, 2024. Title: METHODS FOR TREATING OR PREVENTING ASTHMA BY ADMINISTERING AN IL-4R ANTAGONIST. Applicant: Sanofi Biotechnology. Application EP. The sequence listing filed with the application follows.

SEQUENCE LISTING (275 sequences)

SEQ ID NO: 1 - DNA, 351 bp, synthetic construct
  misc_feature 1..351: note = Synthetic
  source 1..351: mol_type = other DNA
caggtgcagctggtggagtctgggggaggcgtggtccagcctgggaggtccctgagactctcctgtgcagcctctggattcaccttccgctcttatggcatgcactgggtccgccaggctccaggcaaggggctggagtgggtggcggtcatatcatatgatggaagtaataaatattatatagactccgtgaagggccgattcaccatctccagagacaattccaagaacacgctgaatctgcaaatgaacagcctgagacttgaggacacggctgtatattactgtgcgaaagaggggagggggggatttgactactggggccagggaatcccggtcaccgtctcctca

SEQ ID NO: 2 - protein, 117 aa, synthetic construct
  REGION 1..117: note = Synthetic
QVQLVESGGGVVQPGRSLRLSCAASGFTFRSYGMHWVRQAPGKGLEWVAVISYDGSNKYYIDSVKGRFTISRDNSKNTLNLQMNSLRLEDTAVYYCAKEGRGGFDYWGQGIPVTVSS

SEQ ID NO: 3 - DNA, 24 bp, synthetic construct
  misc_feature 1..24: note = Synthetic
  source 1..24: mol_type = other DNA
ggattcaccttccgctcttatggc

SEQ ID NO: 4 - protein, 8 aa, synthetic construct
  REGION 1..8: note = Synthetic
GFTFRSYG

SEQ ID NO: 5 - DNA, 24 bp, synthetic construct
  misc_feature 1..24: note = Synthetic
  source 1..24: mol_type = other DNA
atatcatatgatggaagtaataaa

SEQ ID NO: 6 - protein, 8 aa, synthetic construct
  REGION 1..8: note = Synthetic
ISYDGSNK

SEQ ID NO: 7 - DNA, 30 bp, synthetic construct
  misc_feature 1..30: note = Synthetic
  source 1..30: mol_type = other DNA
gcgaaagaggggagggggggatttgactac

SEQ ID NO: 8 - protein, 10 aa, synthetic construct
  REGION 1..10: note = Synthetic
AKEGRGGFDY

SEQ ID NO: 9 - DNA, 324 bp, synthetic construct
  misc_feature 1..324: note = Synthetic
  source 1..324: mol_type = other DNA
gacatccagatgacccagtctccatcctcactgtctgcatctgtaggagacagagtcaccatcacttgtcgggcgagtcaggtcataaacaattatttagcctggtttcagcagaaaccagggaaagtccctaagtccctgatccatgctgcatccagtttacaaagtggggtcccatcaaagttcagcggcagtggatctgggacagatttcactctcaccatcagcagcctgcagcctgaagattttgcaacttattactgccaacagtataatagtcacccgtggacgttcggccaagggaccaaggtggaaatcaaacga

SEQ ID NO: 10 - protein, 108 aa, synthetic construct
  REGION 1..108: note = Synthetic
DIQMTQSPSSLSASVGDRVTITCRASQVINNYLAWFQQKPGKVPKSLIHAASSLQSGVPSKFSGSGSGTDFTLTISSLQPEDFATYYCQQYNSHPWTFGQGTKVEIKR

SEQ ID NO: 11 - DNA, 18 bp, synthetic construct
  misc_feature 1..18: note = Synthetic
  source 1..18: mol_type = other DNA
caggtcataaacaattat

SEQ ID NO: 12 - protein, 6 aa, synthetic construct
  REGION 1..6: note = Synthetic
QVINNY

SEQ ID NO: 13-14 - skipped (2 entries)

SEQ ID NO: 15 - DNA, 27 bp, synthetic construct
  misc_feature 1..27: note = Synthetic
  source 1..27: mol_type = other DNA
caacagtataatagtcacccgtggacg

SEQ ID NO: 16 - protein, 9 aa, synthetic construct
  REGION 1..9: note = Synthetic
QQYNSHPWT

SEQ ID NO: 17 - DNA, 351 bp, synthetic construct
  misc_feature 1..351: note = Synthetic
  source 1..351: mol_type = other DNA
caggtgcagctggtggagtctgggggaggcgtggtccagcctgggaggtccctgagactctcctgtgcagcctctggattcaccttccgctcttatggcatgcactgggtccgccaggctccaggcaaggggctggagtgggtggcggtcatatcatatgatggaagtaataaatattatatagactccgtgaagggccgattcaccatctccagagacaattccaagaacacgctgaatctgcaaatgaacagcctgagacttgaggacacggctgtatattactgtgcgaaagaggggagggggggatttgactactggggccagggaaccctggtcaccgtctcctca

SEQ ID NO: 18 - protein, 117 aa, synthetic construct
  REGION 1..117: note = Synthetic
QVQLVESGGGVVQPGRSLRLSCAASGFTFRSYGMHWVRQAPGKGLEWVAVISYDGSNKYYIDSVKGRFTISRDNSKNTLNLQMNSLRLEDTAVYYCAKEGRGGFDYWGQGTLVTVSS

SEQ ID NO: 19 - DNA, 321 bp, synthetic construct
  misc_feature 1..321: note = Synthetic
  source 1..321: mol_type = other DNA
gacatccagatgacccagtctccatcctcactgtctgcatctgtaggagacagagtcaccatcacttgtcgggcgagtcaggtcataaacaattatttagcctggtttcagcagaaaccagggaaagtccctaagtccctgatccatgctgcatccagtttacaaagtggggtcccatcaaagttcagcggcagtggatctgggacagatttcactctcaccatcagcagcctgcagcctgaagattttgcaacttattactgccaacagtataatagtcacccgtggacgttcggccaagggaccaaggtggaaatcaaa

SEQ ID NO: 20 - protein, 107 aa, synthetic construct
  REGION 1..107: note = Synthetic
DIQMTQSPSSLSASVGDRVTITCRASQVINNYLAWFQQKPGKVPKSLIHAASSLQSGVPSKFSGSGSGTDFTLTISSLQPEDFATYYCQQYNSHPWTFGQGTKVEIK

SEQ ID NO: 21 - DNA, 351 bp, synthetic construct
  misc_feature 1..351: note = Synthetic
  source 1..351: mol_type = other DNA
caggtgcagctggtggagtctgggggaggcgtggtccagcctgggaggtccctgagactctcctgtgcagcctctggattcaccttccgctcttatggcatgcactgggtccgccaggctccaggcaaggggctggagtgggtggcagttatatcatatgatggaagtaataaatactatgcagactccgtgaagggccgattcaccatctccagagacaattccaagaacacgctgtatctgcaaatgaacagcctgagagctgaggacacggctgtgtattactgtgcgaaagaggggagggggggatttgactactggggccagggaaccctggtcaccgtctcctca

SEQ ID NO: 22 - protein, 117 aa, synthetic construct
  REGION 1..117: note = Synthetic
QVQLVESGGGVVQPGRSLRLSCAASGFTFRSYGMHWVRQAPGKGLEWVAVISYDGSNKYYADSVKGRFTISRDNSKNTLYLQMNSLRAEDTAVYYCAKEGRGGFDYWGQGTLVTVSS

SEQ ID NO: 23 - DNA, 322 bp, synthetic construct
  misc_feature 1..322: note = Synthetic
  source 1..322: mol_type = other DNA
gacatccagatgacccagtctccatcctcactgtctgcatctgtaggagacagagtcaccatcacttgtcgggcgagtcaggtcataaacaattatttagcctggtttcagcagaaaccagggaaagcccctaagtccctgatctatgctgcatccagtttgcaaagtggggtcccatcaaggttcagcggcagtggatctgggacagatttcactctcaccatcagcagcctgcagcctgaagattttgcaacttattactgccaacagtataatagtcacccgtggacgttcggccaagggaccaaggtggaaatcaaac

SEQ ID NO: 24 - protein, 107 aa, synthetic construct
  REGION 1..107: note = Synthetic
DIQMTQSPSSLSASVGDRVTITCRASQVINNYLAWFQQKPGKAPKSLIYAASSLQSGVPSRFSGSGSGTDFTLTISSLQPEDFATYYCQQYNSHPWTFGQGTKVEIK

SEQ ID NO: 25 - DNA, 351 bp, synthetic construct
  misc_feature 1..351: note = Synthetic
  source 1..351: mol_type = other DNA
caggtgcagctggtggagtctgggggaggcgtggtccagcctgggaggtccctgagactctcctgtgcagcctctggattcaccttcagaagctatggcatacactgggtccgccaggctccaggcaaggggctggagtgggtggcagttatatcatatgatggaagtaataaatactatgcagactccgtgaagggccgattcaccatctccagagacaattccaagaacacactgtatctgcaaatgaacagcctgataactgaggacacggctgtgtattattgtgtgaaagaggggaggggggggtttgactactggggccagggaaccacggtcaccgtctcctca

SEQ ID NO: 26 - protein, 117 aa, synthetic construct
  REGION 1..117: note = Synthetic
QVQLVESGGGVVQPGRSLRLSCAASGFTFRSYGIHWVRQAPGKGLEWVAVISYDGSNKYYADSVKGRFTISRDNSKNTLYLQMNSLITEDTAVYYCVKEGRGGFDYWGQGTTVTVSS

SEQ ID NO: 27 - DNA, 24 bp, synthetic construct
  misc_feature 1..24: note = Synthetic
  source 1..24: mol_type = other DNA
ggattcaccttcagaagctatggc

SEQ ID NO: 28 - protein, 8 aa, synthetic construct
  REGION 1..8: note = Synthetic
GFTFRSYG

SEQ ID NO: 29 - DNA, 24 bp, synthetic construct
  misc_feature 1..24: note = Synthetic
  source 1..24: mol_type = other DNA
atatcatatgatggaagtaataaa

SEQ ID NO: 30 - protein, 8 aa, synthetic construct
  REGION 1..8: note = Synthetic
ISYDGSNK

SEQ ID NO: 31 - DNA, 30 bp, synthetic construct
  misc_feature 1..30: note = Synthetic
  source 1..30: mol_type = other DNA
gtgaaagaggggaggggggggtttgactac

SEQ ID NO: 32 - protein, 10 aa, synthetic construct
  REGION 1..10: note = Synthetic
VKEGRGGFDY

SEQ ID NO: 33 - DNA, 324 bp, synthetic construct
  misc_feature 1..324: note = Synthetic
  source 1..324: mol_type = other DNA
gacatccagatgacccagtctccatcctcactgtctgcatctgtaggagacagagtcaccatcacttgtcgggcgagtcaggtcattaataattatttagcctggtttcagcagaaaccagggaaagtccctaagtccctgatccatgctgcatccagtttgcaaagaggggtcccatcaaagttcagcggcagtggatctgggacagatttcactctcaccatcaacagcctgcagcctgaagattttgcaacttattactgccaacaatataatagttacccgtggacgttcggccaagggaccaaggtggaaatcaaacga

SEQ ID NO: 34 - protein, 108 aa, synthetic construct
  REGION 1..108: note = Synthetic
DIQMTQSPSSLSASVGDRVTITCRASQVINNYLAWFQQKPGKVPKSLIHAASSLQRGVPSKFSGSGSGTDFTLTINSLQPEDFATYYCQQYNSYPWTFGQGTKVEIKR

SEQ ID NO: 35 - DNA, 18 bp, synthetic construct
  misc_feature 1..18: note = Synthetic
  source 1..18: mol_type = other DNA
caggtcattaataattat

SEQ ID NO: 36 - protein, 6 aa, synthetic construct
  REGION 1..6: note = Synthetic
QVINNY

SEQ ID NO: 37-38 - skipped (2 entries)

SEQ ID NO: 39 - DNA, 27 bp, synthetic construct
  misc_feature 1..27: note = Synthetic
  source 1..27: mol_type = other DNA
caacaatataatagttacccgtggacg

SEQ ID NO: 40 - protein, 9 aa, synthetic construct
  REGION 1..9: note = Synthetic
QQYNSYPWT

SEQ ID NO: 41 - DNA, 351 bp, synthetic construct
  misc_feature 1..351: note = Synthetic
  source 1..351: mol_type = other DNA
caggtgcagctggtggagtctgggggaggcgtggtccagcctgggaggtccctgagactctcctgtgcagcctctggattcaccttcagaagctatggcatacactgggtccgccaggctccaggcaaggggctggagtgggtggcagttatatcatatgatggaagtaataaatactatgcagactccgtgaagggccgattcaccatctccagagacaattccaagaacacactgtatctgcaaatgaacagcctgataactgaggacacggctgtgtattattgtgtgaaagaggggaggggggggtttgactactggggccagggaaccctggtcaccgtctcctca

SEQ ID NO: 42 - protein, 117 aa, synthetic construct
  REGION 1..117: note = Synthetic
QVQLVESGGGVVQPGRSLRLSCAASGFTFRSYGIHWVRQAPGKGLEWVAVISYDGSNKYYADSVKGRFTISRDNSKNTLYLQMNSLITEDTAVYYCVKEGRGGFDYWGQGTLVTVSS

SEQ ID NO: 43 - DNA, 321 bp, synthetic construct
  misc_feature 1..321: note = Synthetic
  source 1..321: mol_type = other DNA
gacatccagatgacccagtctccatcctcactgtctgcatctgtaggagacagagtcaccatcacttgtcgggcgagtcaggtcattaataattatttagcctggtttcagcagaaaccagggaaagtccctaagtccctgatccatgctgcatccagtttgcaaagaggggtcccatcaaagttcagcggcagtggatctgggacagatttcactctcaccatcaacagcctgcagcctgaagattttgcaacttattactgccaacaatataatagttacccgtggacgttcggccaagggaccaaggtggaaatcaaa

SEQ ID NO: 44 - protein, 107 aa, synthetic construct
  REGION 1..107: note = Synthetic
DIQMTQSPSSLSASVGDRVTITCRASQVINNYLAWFQQKPGKVPKSLIHAASSLQRGVPSKFSGSGSGTDFTLTINSLQPEDFATYYCQQYNSYPWTFGQGTKVEIK

SEQ ID NO: 45 - DNA, 351 bp, synthetic construct
  misc_feature 1..351: note = Synthetic
  source 1..351: mol_type = other DNA
caggtgcagctggtggagtctgggggaggcgtggtccagcctgggaggtccctgagactctcctgtgcagcctctggattcaccttcagaagctatggcatgcactgggtccgccaggctccaggcaaggggctggagtgggtggcagttatatcatatgatggaagtaataaatactatgcagactccgtgaagggccgattcaccatctccagagacaattccaagaacacgctgtatctgcaaatgaacagcctgagagctgaggacacggctgtgtattactgtgtgaaagaggggaggggggggtttgactactggggccagggaaccctggtcaccgtctcctca

SEQ ID NO: 46 - protein, 117 aa, synthetic construct
  REGION 1..117: note = Synthetic
QVQLVESGGGVVQPGRSLRLSCAASGFTFRSYGMHWVRQAPGKGLEWVAVISYDGSNKYYADSVKGRFTISRDNSKNTLYLQMNSLRAEDTAVYYCVKEGRGGFDYWGQGTLVTVSS

SEQ ID NO: 47 - DNA, 322 bp, synthetic construct
  misc_feature 1..322: note = Synthetic
  source 1..322: mol_type = other DNA
gacatccagatgacccagtctccatcctcactgtctgcatctgtaggagacagagtcaccatcacttgtcgggcgagtcaggtcattaataattatttagcctggtttcagcagaaaccagggaaagcccctaagtccctgatctatgctgcatccagtttgcaaagtggggtcccatcaaggttcagcggcagtggatctgggacagatttcactctcaccatcagcagcctgcagcctgaagattttgcaacttattactgccaacaatataatagttacccgtggacgttcggccaagggaccaaggtggaaatcaaac

SEQ ID NO: 48 - protein, 107 aa, synthetic construct
  REGION 1..107: note = Synthetic
DIQMTQSPSSLSASVGDRVTITCRASQVINNYLAWFQQKPGKAPKSLIYAASSLQSGVPSRFSGSGSGTDFTLTISSLQPEDFATYYCQQYNSYPWTFGQGTKVEIK

SEQ ID NO: 49 - DNA, 375 bp, synthetic construct
  misc_feature 1..375: note = Synthetic
  source 1..375: mol_type = other DNA
caggtgcagctggtggagtctgggggaggcttggaacagccgggggggtccttgagactctcctgtgcaggctctggattcacgtttagagactatgccatgacctgggtccgccaggctccagggaaggggctggagtgggtcgcatcgattagtggttccggtggtaacacatacttcgcagactccgtgaagggccggttcaccatctccagagacaattccaagaacacgctgtatctgcaaatgaacagcctgagagccgaggacacggccgtatattactgtgcgaaagatcgactctctataacaattcgcccacgctattatggtttggacgtctggggccaagggtccacggtcaccgtctcctca

SEQ ID NO: 50 - protein, 125 aa, synthetic construct
  REGION 1..125: note = Synthetic
QVQLVESGGGLEQPGGSLRLSCAGSGFTFRDYAMTWVRQAPGKGLEWVASISGSGGNTYFADSVKGRFTISRDNSKNTLYLQMNSLRAEDTAVYYCAKDRLSITIRPRYYGLDVWGQGSTVTVSS

SEQ ID NO: 51 - DNA, 24 bp, synthetic construct
  misc_feature 1..24: note = Synthetic
  source 1..24: mol_type = other DNA
ggattcacgtttagagactatgcc

SEQ ID NO: 52 - protein, 8 aa, synthetic construct
  REGION 1..8: note = Synthetic
GFTFRDYA

SEQ ID NO: 53 - DNA, 24 bp, synthetic construct
  misc_feature 1..24: note = Synthetic
  source 1..24: mol_type = other DNA
attagtggttccggtggtaacaca

SEQ ID NO: 54 - protein, 8 aa, synthetic construct
  REGION 1..8: note = Synthetic
ISGSGGNT

SEQ ID NO: 55 - DNA, 54 bp, synthetic construct
  misc_feature 1..54: note = Synthetic
  source 1..54: mol_type = other DNA
gcgaaagatcgactctctataacaattcgcccacgctattatggtttggacgtc

SEQ ID NO: 56 - protein, 18 aa, synthetic construct
  REGION 1..18: note = Synthetic
AKDRLSITIRPRYYGLDV

SEQ ID NO: 57 - DNA, 324 bp, synthetic construct
  misc_feature 1..324: note = Synthetic
  source 1..324: mol_type = other DNA
gacatccagatgacccagtctccatcctcactgtctgcatctgttggagacagagtcaccatcacttgtcgggcgagtcaggccattaacaatcatttagcctggtttcagcagaaaccagggaaagcccctaagtccctgatctttgctgtatccagtttgcaaagtggggtcccatcaaagttcagcggcagtggatctgggacagacttcactctcaccatcagcagcctgcagcctgaagattttgcaacttattactgccaacagtataatagttacccgtggacgttcggccaagggaccaaggtggaaatcaaacga

SEQ ID NO: 58 - protein, 108 aa, synthetic construct
  REGION 1..108: note = Synthetic
DIQMTQSPSSLSASVGDRVTITCRASQAINNHLAWFQQKPGKAPKSLIFAVSSLQSGVPSKFSGSGSGTDFTLTISSLQPEDFATYYCQQYNSYPWTFGQGTKVEIKR

SEQ ID NO: 59 - DNA, 18 bp, synthetic construct
  misc_feature 1..18: note = Synthetic
  source 1..18: mol_type = other DNA
caggccattaacaatcat

SEQ ID NO: 60 - protein, 6 aa, synthetic construct
  REGION 1..6: note = Synthetic
QAINNH

SEQ ID NO: 61-62 - skipped (2 entries)

SEQ ID NO: 63 - DNA, 27 bp, synthetic construct
  misc_feature 1..27: note = Synthetic
  source 1..27: mol_type = other DNA
caacagtataatagttacccgtggacg

SEQ ID NO: 64 - protein, 9 aa, synthetic construct
  REGION 1..9: note = Synthetic
QQYNSYPWT

SEQ ID NO: 65 - DNA, 372 bp, synthetic construct
  misc_feature 1..372: note = Synthetic
  source 1..372: mol_type = other DNA
gaggtgcagctggtggagtctgggggaggcttggaacagccgggggggtccttgagactctcctgtgcaggctctggattcacgtttagagactatgccatgacctgggtccgccaggctccagggaaggggctggagtgggtcgcatcgattagtggttccggtggtaacacatacttcgcagactccgtgaagggccggttcaccatctccagagacaattccaagaacacgctgtatctgcaaatgaacagcctgagagccgaggacacggccgtatattactgtgcgaaagatcgactctctataacaattcgcccacgctattatggtttggacgtctggggccaagggaccacggtcaccgtctcc

SEQ ID NO: 66 - protein, 124 aa, synthetic construct
  REGION 1..124: note = Synthetic
EVQLVESGGGLEQPGGSLRLSCAGSGFTFRDYAMTWVRQAPGKGLEWVASISGSGGNTYFADSVKGRFTISRDNSKNTLYLQMNSLRAEDTAVYYCAKDRLSITIRPRYYGLDVWGQGTTVTVS

SEQ ID NO: 67 - DNA, 321 bp, synthetic construct
  misc_feature 1..321: note = Synthetic
  source 1..321: mol_type = other DNA
gacatccagatgacccagtctccatcctcactgtctgcatctgttggagacagagtcaccatcacttgtcgggcgagtcaggccattaacaatcatttagcctggtttcagcagaaaccagggaaagcccctaagtccctgatctttgctgtatccagtttgcaaagtggggtcccatcaaagttcagcggcagtggatctgggacagacttcactctcaccatcagcagcctgcagcctgaagattttgcaacttattactgccaacagtataatagttacccgtggacgttcggccaagggaccaaggtggaaatcaaa

SEQ ID NO: 68 - protein, 107 aa, synthetic construct
  REGION 1..107: note = Synthetic
DIQMTQSPSSLSASVGDRVTITCRASQAINNHLAWFQQKPGKAPKSLIFAVSSLQSGVPSKFSGSGSGTDFTLTISSLQPEDFATYYCQQYNSYPWTFGQGTKVEIK

SEQ ID NO: 69 - DNA, 373 bp, synthetic construct
  misc_feature 1..373: note = Synthetic
  source 1..373: mol_type = other DNA
gaggtgcagctggtggagtctgggggaggcttggtacagcctggggggtccctgagactctcctgtgcagcctctggattcacgtttagagactatgccatgagctgggtccgccaggctccagggaaggggctggagtgggtctcagctattagtggttccggtggtaacacatactacgcagactccgtgaagggccggttcaccatctccagagacaattccaagaacacgctgtatctgcaaatgaacagcctgagagccgaggacacggccgtatattactgtgcgaaagatcgactctctataacaattcgcccacgctattatggtttggacgtctggggccaagggaccacggtcaccgtctcct

SEQ ID NO: 70 - protein, 124 aa, synthetic construct
  REGION 1..124: note = Synthetic
EVQLVESGGGLVQPGGSLRLSCAASGFTFRDYAMSWVRQAPGKGLEWVSAISGSGGNTYYADSVKGRFTISRDNSKNTLYLQMNSLRAEDTAVYYCAKDRLSITIRPRYYGLDVWGQGTTVTVS

SEQ ID NO: 71 - DNA, 322 bp, synthetic construct
  misc_feature 1..322: note = Synthetic
  source 1..322: mol_type = other DNA
gacatccagatgacccagtctccatcctcactgtctgcatctgtaggagacagagtcaccatcacttgtcgggcgagtcaggccattaacaatcatttagcctggtttcagcagaaaccagggaaagcccctaagtccctgatctatgctgtatccagtttgcaaagtggggtcccatcaaggttcagcggcagtggatctgggacagatttcactctcaccatcagcagcctgcagcctgaagattttgcaacttattactgccaacagtataatagttacccgtggacgttcggccaagggaccaaggtggaaatcaaac

SEQ ID NO: 72 - protein, 107 aa, synthetic construct
  REGION 1..107: note = Synthetic
DIQMTQSPSSLSASVGDRVTITCRASQAINNHLAWFQQKPGKAPKSLIYAVSSLQSGVPSRFSGSGSGTDFTLTISSLQPEDFATYYCQQYNSYPWTFGQGTKVEIK

SEQ ID NO: 73 - DNA, 375 bp, synthetic construct; identical to SEQ ID NO: 49
  misc_feature 1..375: note = Synthetic
  source 1..375: mol_type = other DNA

SEQ ID NO: 74 - protein, 125 aa, synthetic construct; identical to SEQ ID NO: 50
  REGION 1..125: note = Synthetic

SEQ ID NO: 75 - DNA, 24 bp, synthetic construct
  misc_feature 1..24: note = Synthetic
  source 1..24: mol_type = other DNA
ggattcacgtttagagactatgcc

SEQ ID NO: 76 - protein, 8 aa, synthetic construct
  REGION 1..8: note = Synthetic
GFTFRDYA

SEQ ID NO: 77 - DNA, 24 bp, synthetic construct
  misc_feature 1..24: note = Synthetic
  source 1..24: mol_type = other DNA
attagtggttccggtggtaacaca

SEQ ID NO: 78 - protein, 8 aa, synthetic construct
  REGION 1..8: note = Synthetic
ISGSGGNT

SEQ ID NO: 79 - DNA, 54 bp, synthetic construct; identical to SEQ ID NO: 55
  misc_feature 1..54: note = Synthetic
  source 1..54: mol_type = other DNA

SEQ ID NO: 80 - protein, 18 aa, synthetic construct
  REGION 1..18: note = Synthetic
AKDRLSITIRPRYYGLDV

SEQ ID NO: 81 - DNA, 339 bp, synthetic construct
  misc_feature 1..339: note = Synthetic
  source 1..339: mol_type = other DNA
gaaatagtgttgacgcagtctccactctccctgcccgtcacccctggagagccggcctccatctcctgcaggtctagtcagagcctcctgtatagtattggatacaactatttggattggtacctgcagaagtcagggcagtctccacagctccttatctatttgggttctaatcgggcctccggggtccctgacaggttcagtggcagtggatcaggcacagattttacactgaaaatcagcagagtggaggctgaggatgttgggttttattactgcatgcaagctctacaaactccgtacacttttggcccggggaccaagctggagatcaaacga

SEQ ID NO: 82 - protein, 113 aa, synthetic construct
  REGION 1..113: note = Synthetic
EIVLTQSPLSLPVTPGEPASISCRSSQSLLYSIGYNYLDWYLQKSGQSPQLLIYLGSNRASGVPDRFSGSGSGTDFTLKISRVEAEDVGFYYCMQALQTPYTFGPGTKLEIKR

SEQ ID NO: 83 - DNA, 33 bp, synthetic construct
  misc_feature 1..33: note = Synthetic
  source 1..33: mol_type = other DNA
cagagcctcctgtatagtattggatacaactat

SEQ ID NO: 84 - protein, 11 aa, synthetic construct
  REGION 1..11: note = Synthetic
QSLLYSIGYNY

SEQ ID NO: 85-86 - skipped (2 entries)

SEQ ID NO: 87 - DNA, 27 bp, synthetic construct
  misc_feature 1..27: note = Synthetic
  source 1..27: mol_type = other DNA
atgcaagctctacaaactccgtacact

SEQ ID NO: 88 - protein, 9 aa, synthetic construct
  REGION 1..9: note = Synthetic
MQALQTPYT

SEQ ID NO: 89 - DNA, 372 bp, synthetic construct; identical to SEQ ID NO: 65
  misc_feature 1..372: note = Synthetic
  source 1..372: mol_type = other DNA

SEQ ID NO: 90 - protein, 124 aa, synthetic construct; identical to SEQ ID NO: 66
  REGION 1..124: note = Synthetic

SEQ ID NO: 91 - DNA, 336 bp, synthetic construct
  misc_feature 1..336: note = Synthetic
  source 1..336: mol_type = other DNA
gatattgtgatgactcagtctccactctccctgcccgtcacccctggagagccggcctccatctcctgcaggtctagtcagagcctcctgtatagtattggatacaactatttggattggtacctgcagaagtcagggcagtctccacagctccttatctatttgggttctaatcgggcctccggggtccctgacaggttcagtggcagtggatcaggcacagattttacactgaaaatcagcagagtggaggctgaggatgttgggttttattactgcatgcaagctctacaaactccgtacacttttggcccggggaccaagctggagatcaaa

SEQ ID NO: 92 - protein, 112 aa, synthetic construct
  REGION 1..112: note = Synthetic
DIVMTQSPLSLPVTPGEPASISCRSSQSLLYSIGYNYLDWYLQKSGQSPQLLIYLGSNRASGVPDRFSGSGSGTDFTLKISRVEAEDVGFYYCMQALQTPYTFGPGTKLEIK

SEQ ID NO: 93 - DNA, 373 bp, synthetic construct; identical to SEQ ID NO: 69
  misc_feature 1..373: note = Synthetic
  source 1..373: mol_type = other DNA

SEQ ID NO: 94 - protein, 124 aa, synthetic construct; identical to SEQ ID NO: 70
  REGION 1..124: note = Synthetic

SEQ ID NO: 95 - DNA, 337 bp, synthetic construct
  misc_feature 1..337: note = Synthetic
  source 1..337: mol_type = other DNA
gatattgtgatgactcagtctccactctccctgcccgtcacccctggagagccggcctccatctcctgcaggtctagtcagagcctcctgtatagtattggatacaactatttggattggtacctgcagaagccagggcagtctccacagctcctgatctatttgggttctaatcgggcctccggggtccctgacaggttcagtggcagtggatcaggcacagattttacactgaaaatcagcagagtggaggctgaggatgttggggtttattactgcatgcaagctctacaaactccgtacacttttggccaggggaccaagctggagatcaaac

SEQ ID NO: 96 - protein, 112 aa, synthetic construct
  REGION 1..112: note = Synthetic
DIVMTQSPLSLPVTPGEPASISCRSSQSLLYSIGYNYLDWYLQKPGQSPQLLIYLGSNRASGVPDRFSGSGSGTDFTLKISRVEAEDVGVYYCMQALQTPYTFGQGTKLEIK

SEQ ID NO: 97 - DNA, 375 bp, synthetic construct
  misc_feature 1..375: note = Synthetic
  source 1..375: mol_type = other DNA
caggtgcagctggtggagtctgagggactcttggaacagcctggggggtccctgagactctcctgtgcagcctctggattcaactttagagactttgccatgacctgggtccgccaggctccagggaaggggctggagtgggtctcatctattagtggtagtggtagtaatacatactacgcagactccgtgaagggccggttcaccatctccagagacaattccaaccacacgctgtatctgcgaatgaacagcctgagagccgaagacacggccgtgtattactgtgcgaaagatcgactctctataacaattcgcccacgctattacggtctggacgtctggggccaagggtccacggtcaccgtctcctca

SEQ ID NO: 98 - protein, 125 aa, synthetic construct
  REGION 1..125: note = Synthetic
QVQLVESEGLLEQPGGSLRLSCAASGFNFRDFAMTWVRQAPGKGLEWVSSISGSGSNTYYADSVKGRFTISRDNSNHTLYLRMNSLRAEDTAVYYCAKDRLSITIRPRYYGLDVWGQGSTVTVSS

SEQ ID NO: 99 - DNA, 24 bp, synthetic construct
  misc_feature 1..24: note = Synthetic
  source 1..24: mol_type = other DNA
ggattcaactttagagactttgcc

SEQ ID NO: 100 - protein, 8 aa, synthetic construct
  REGION 1..8: note = Synthetic
GFNFRDFA

SEQ ID NO: 101 - DNA, 24 bp, synthetic construct
  misc_feature 1..24: note = Synthetic
  source 1..24: mol_type = other DNA
attagtggtagtggtagtaataca

SEQ ID NO: 102 - protein, 8 aa, synthetic construct
  REGION 1..8: note = Synthetic
ISGSGSNT

SEQ ID NO: 103 - DNA, 54 bp, synthetic construct
  misc_feature 1..54: note = Synthetic
  source 1..54: mol_type = other DNA
gcgaaagatcgactctctataacaattcgcccacgctattacggtctggacgtc

SEQ ID NO: 104 - protein, 18 aa, synthetic construct
  REGION 1..18: note = Synthetic
AKDRLSITIRPRYYGLDV

SEQ ID NO: 105 - DNA, 324 bp, synthetic construct
  misc_feature 1..324: note = Synthetic
  source 1..324: mol_type = other DNA
gacatccagatgacccagtctccatcctccctgtctgcatctgtaggagacagagtcaccatcacttgccgggcgagtcaggacattagcaattattttgcctggtatcagcagaagccagggaaagttcctaagctcctgatctttgctgcatccactttgcatccaggggtcccatctcggttcagtggcagtggatctgggacagatttcactctcaccattcgcagcctgcagcctgaagatgttgcaacttattactgtcaaaaatatgacagtgccccgtacacttttggccaggggaccaaggtggaaatcaaacga

SEQ ID NO: 106 - protein, 108 aa, synthetic construct
  REGION 1..108: note = Synthetic
DIQMTQSPSSLSASVGDRVTITCRASQDISNYFAWYQQKPGKVPKLLIFAASTLHPGVPSRFSGSGSGTDFTLTIRSLQPEDVATYYCQKYDSAPYTFGQGTKVEIKR

SEQ ID NO: 107 - DNA, 18 bp, synthetic construct
  misc_feature 1..18: note = Synthetic
  source 1..18: mol_type = other DNA
caggacattagcaattat

SEQ ID NO: 108 - protein, 6 aa, synthetic construct
  REGION 1..6: note = Synthetic
QDISNY

SEQ ID NO: 109-110 - skipped (2 entries)

SEQ ID NO: 111 - DNA, 27 bp, synthetic construct
  misc_feature 1..27: note = Synthetic
  source 1..27: mol_type = other DNA
caaaaatatgacagtgccccgtacact

SEQ ID NO: 112 - protein, 9 aa, synthetic construct
  REGION 1..9: note = Synthetic
QKYDSAPYT

SEQ ID NO: 113 - DNA, 372 bp, synthetic construct
  misc_feature 1..372: note = Synthetic
  source 1..372: mol_type = other DNA
gaggtgcagctggtggagtctgagggactcttggaacagcctggggggtccctgagactctcctgtgcagcctctggattcaactttagagactttgccatgacctgggtccgccaggctccagggaaggggctggagtgggtctcatctattagtggtagtggtagtaatacatactacgcagactccgtgaagggccggttcaccatctccagagacaattccaaccacacgctgtatctgcgaatgaacagcctgagagccgaagacacggccgtgtattactgtgcgaaagatcgactctctataacaattcgcccacgctattacggtctggacgtctggggccaagggaccacggtcaccgtctcc

SEQ ID NO: 114 - protein, 124 aa, synthetic construct
  REGION 1..124: note = Synthetic
EVQLVESEGLLEQPGGSLRLSCAASGFNFRDFAMTWVRQAPGKGLEWVSSISGSGSNTYYADSVKGRFTISRDNSNHTLYLRMNSLRAEDTAVYYCAKDRLSITIRPRYYGLDVWGQGTTVTVS

SEQ ID NO: 115 - DNA, 321 bp, synthetic construct
  misc_feature 1..321: note = Synthetic
  source 1..321: mol_type = other DNA
gacatccagatgacccagtctccatcctccctgtctgcatctgtaggagacagagtcaccatcacttgccgggcgagtcaggacattagcaattattttgcctggtatcagcagaagccagggaaagttcctaagctcctgatctttgctgcatccactttgcatccaggggtcccatctcggttcagtggcagtggatctgggacagatttcactctcaccattcgcagcctgcagcctgaagatgttgcaacttattactgtcaaaaatatgacagtgccccgtacacttttggccaggggaccaagctggagatcaaa

SEQ ID NO: 116 - protein, 107 aa, synthetic construct
  REGION 1..107: note = Synthetic
DIQMTQSPSSLSASVGDRVTITCRASQDISNYFAWYQQKPGKVPKLLIFAASTLHPGVPSRFSGSGSGTDFTLTIRSLQPEDVATYYCQKYDSAPYTFGQGTKLEIK

SEQ ID NO: 117 - DNA, 373 bp, synthetic construct
  misc_feature 1..373: note = Synthetic
  source 1..373: mol_type = other DNA
gaggtgcagctggtggagtctgggggaggcttggtacagcctggggggtccctgagactctcctgtgcagcctctggattcaactttagagactttgccatgagctgggtccgccaggctccagggaaggggctggagtgggtctcagctattagtggtagtggtagtaatacatactacgcagactccgtgaagggccggttcaccatctccagagacaattccaagaacacgctgtatctgcaaatgaacagcctgagagccgaggacacggccgtatattactgtgcgaaagatcgactctctataacaattcgcccacgctattacggtctggacgtctggggccaagggaccacggtcaccgtctcct

SEQ ID NO: 118 - protein, 124 aa, synthetic construct
  REGION 1..124: note = Synthetic
EVQLVESGGGLVQPGGSLRLSCAASGFNFRDFAMSWVRQAPGKGLEWVSAISGSGSNTYYADSVKGRFTISRDNSKNTLYLQMNSLRAEDTAVYYCAKDRLSITIRPRYYGLDVWGQGTTVTVS

SEQ ID NO: 119 - DNA, 322 bp, synthetic construct
  misc_feature 1..322: note = Synthetic
  source 1..322: mol_type = other DNA
gacatccagatgacccagtctccatcctccctgtctgcatctgtaggagacagagtcaccatcacttgccgggcgagtcaggacattagcaattatttagcctggtatcagcagaaaccagggaaagttcctaagctcctgatctatgctgcatccactttgcaatcaggggtcccatctcggttcagtggcagtggatctgggacagatttcactctcaccatcagcagcctgcagcctgaagatgttgcaacttattactgtcaaaaatatgacagtgccccgtacacttttggccaggggaccaagctggagatcaaac

SEQ ID NO: 120 - protein, 107 aa, synthetic construct
  REGION 1..107: note = Synthetic
DIQMTQSPSSLSASVGDRVTITCRASQDISNYLAWYQQKPGKVPKLLIYAASTLQSGVPSRFSGSGSGTDFTLTISSLQPEDVATYYCQKYDSAPYTFGQGTKLEIK

SEQ ID NO: 121 - DNA, 357 bp, synthetic construct
  misc_feature 1..357: note = Synthetic
  source 1..357: mol_type = other DNA
caggtgcagctggtggagtctgggggaggcttggtacagcctggggggtccctgagactctcctgtgtagcttctggattcacccttaacaactttgtcatgaactgggtccgccaggttccagggaagggactggagtgggtctcttttattagtgctagtggtggtagtatatactacgcagactccgtgaagggccggttcaccatctccagagacacttccaagaacacattatatctgcaaatgaacagcctgagagccgacgacacggccgtctattactgtgcgaaatccccgtataactggaacccctttgactattggggccagggaaccacggtcaccgtctcctca

SEQ ID NO: 122 - protein, 119 aa, synthetic construct
  REGION 1..119: note = Synthetic
QVQLVESGGGLVQPGGSLRLSCVASGFTLNNFVMNWVRQVPGKGLEWVSFISASGGSIYYADSVKGRFTISRDTSKNTLYLQMNSLRADDTAVYYCAKSPYNWNPFDYWGQGTTVTVSS

SEQ ID NO: 123 - DNA, 24 bp, synthetic construct
  misc_feature 1..24: note = Synthetic
  source 1..24: mol_type = other DNA
ggattcacccttaacaactttgtc

SEQ ID NO: 124 - protein, 8 aa, synthetic construct
  REGION 1..8: note = Synthetic
GFTLNNFV

SEQ ID NO: 125 - DNA, 24 bp, synthetic construct
  misc_feature 1..24: note = Synthetic
  source 1..24: mol_type = other DNA
attagtgctagtggtggtagtata

SEQ ID NO: 126 - protein, 8 aa, synthetic construct
  REGION 1..8: note = Synthetic
ISASGGSI

SEQ ID NO: 127 - DNA, 36 bp, synthetic construct
  misc_feature 1..36: note = Synthetic
  source 1..36: mol_type = other DNA
gcgaaatccccgtataactggaacccctttgactat

SEQ ID NO: 128 - protein, 12 aa, synthetic construct
  REGION 1..12: note = Synthetic
AKSPYNWNPFDY

SEQ ID NO: 129 - DNA, 327 bp, synthetic construct
  misc_feature 1..327: note = Synthetic
  source 1..327: mol_type = other DNA
gacatccagttgacccagtctccagccaccctgtctgtgtctccaggggaacgagccaccctctcctgcagggccagtctgagtgttagcagcaaattagcctggtaccagcagacacctggccaggctcccagactcctcatctatagtgcctccacccgggccactggtatcccagtcaggttcagtggcagtgggtctgggacagagttcactctcaccatcagcagcctgcagtctgaagattttgcggtttattactgtcagcagtataatcattggcctccgtacacttttggccaggggaccaaggtggagatcaaacga

SEQ ID NO: 130 - protein, 109 aa, synthetic construct
  REGION 1..109: note = Synthetic
DIQLTQSPATLSVSPGERATLSCRASLSVSSKLAWYQQTPGQAPRLLIYSASTRATGIPVRFSGSGSGTEFTLTISSLQSEDFAVYYCQQYNHWPPYTFGQGTKVEIKR

SEQ ID NO: 131 - DNA, 18 bp, synthetic construct
  misc_feature 1..18: note = Synthetic
  source 1..18: mol_type = other DNA
ctgagtgttagcagcaaa

SEQ ID NO: 132 - protein, 6 aa, synthetic construct
  REGION 1..6: note = Synthetic
LSVSSK

SEQ ID NO: 133-134 - skipped (2 entries)

SEQ ID NO: 135 - DNA, 30 bp, synthetic construct
  misc_feature 1..30: note = Synthetic
  source 1..30: mol_type = other DNA
cagcagtataatcattggcctccgtacact

SEQ ID NO: 136 - protein, 10 aa, synthetic construct
  REGION 1..10: note = Synthetic
QQYNHWPPYT

SEQ ID NO: 137 - DNA, 357 bp, synthetic construct
  misc_feature 1..357: note = Synthetic
  source 1..357: mol_type = other DNA
gaggtgcagctggtggagtctgggggaggcttggtacagcctggggggtccctgagactctcctgtgtagcttctggattcacccttaacaactttgtcatgaactgggtccgccaggttccagggaagggactggagtgggtctcttttattagtgctagtggtggtagtatatactacgcagactccgtgaagggccggttcaccatctccagagacacttccaagaacacattatatctgcaaatgaacagcctgagagccgacgacacggccgtctattactgtgcgaaatccccgtataactggaacccctttgactattggggccagggaaccctggtcaccgtctcctca

SEQ ID NO: 138 - protein, 119 aa, synthetic construct
  REGION 1..119: note = Synthetic
EVQLVESGGGLVQPGGSLRLSCVASGFTLNNFVMNWVRQVPGKGLEWVSFISASGGSIYYADSVKGRFTISRDTSKNTLYLQMNSLRADDTAVYYCAKSPYNWNPFDYWGQGTLVTVSS

SEQ ID NO: 139 - DNA, 324 bp, synthetic construct
  misc_feature 1..324: note = Synthetic
  source 1..324: mol_type = other DNA
gaaatagtgatgacgcagtctccagccaccctgtctgtgtctccaggggaacgagccaccctctcctgcagggccagtctgagtgttagcagcaaattagcctggtaccagcagacacctggccaggctcccagactcctcatctatagtgcctccacccgggccactggtatcccagtcaggttcagtggcagtgggtctgggacagagttcactctcaccatcagcagcctgcagtctgaagattttgcggtttattactgtcagcagtataatcattggcctccgtacacttttggccaggggaccaagctggagatcaaa

SEQ ID NO: 140 - protein, 108 aa, synthetic construct
  REGION 1..108: note = Synthetic
EIVMTQSPATLSVSPGERATLSCRASLSVSSKLAWYQQTPGQAPRLLIYSASTRATGIPVRFSGSGSGTEFTLTISSLQSEDFAVYYCQQYNHWPPYTFGQGTKLEIK

SEQ ID NO: 141 - DNA, 357 bp, synthetic construct
  misc_feature 1..357: note = Synthetic
  source 1..357: mol_type = other DNA
gaggtgcagctggtggagtctgggggaggcttggtacagcctggggggtccctgagactctcctgtgcagcctctggattcacccttaacaactttgtcatgagctgggtccgccaggctccagggaaggggctggagtgggtctcagctattagtgctagtggtggtagtatatactacgcagactccgtgaagggccggttcaccatctccagagacaattccaagaacacgctgtatctgcaaatgaacagcctgagagccgaggacacggccgtatattactgtgcgaaatccccgtataactggaacccctttgactattggggccagggaaccctggtcaccgtctcctca

SEQ ID NO: 142 - protein, 119 aa, synthetic construct
  REGION 1..119: note = Synthetic
EVQLVESGGGLVQPGGSLRLSCAASGFTLNNFVMSWVRQAPGKGLEWVSAISASGGSIYYADSVKGRFTISRDNSKNTLYLQMNSLRAEDTAVYYCAKSPYNWNPFDYWGQGTLVTVSS

SEQ ID NO: 143 - DNA, 325 bp, synthetic construct
  misc_feature 1..325: note = Synthetic
  source 1..325: mol_type = other DNA
gaaatagtgatgacgcagtctccagccaccctgtctgtgtctccaggggaaagagccaccctctcctgcagggccagtctgagtgttagcagcaaattagcctggtaccagcagaaacctggccaggctcccaggctcctcatctatagtgcctccaccagggccactggtatcccagccaggttcagtggcagtgggtctgggacagagttcactctcaccatcagcagcctgcagtctgaagattttgcagtttattactgtcagcagtataatcattggcctccgtacacttttggccaggggaccaagctggagatcaaac

SEQ ID NO: 144 - protein, 108 aa, synthetic construct
  REGION 1..108: note = Synthetic
EIVMTQSPATLSVSPGERATLSCRASLSVSSKLAWYQQKPGQAPRLLIYSASTRATGIPARFSGSGSGTEFTLTISSLQSEDFAVYYCQQYNHWPPYTFGQGTKLEIK

SEQ ID NO: 145 - DNA, 375 bp, synthetic construct
  misc_feature 1..375: note = Synthetic
  source 1..375: mol_type = other DNA
caggtgcagctggtggagtctgggggaggcttggaacagccgggggggtccctgagactctcctgtgcaggctctggattcacctttagagactatgccatgacctgggtccgccaggctccagggaagggactggagtgggtctcatctattagtggttccggtggtaacacatactacgcagactccgtgaagggccggttcaccatctccagagacaattccaagaacacgctgtatctgcaaatgaacagcctgagagccgaggacacggccgtatattactgtgcgaaagatcgactctctataacaattcgcccacgctattatggtttggacgtctggggccaagggtccacggtcaccgtctcctca

SEQ ID NO: 146 - protein, 125 aa, synthetic construct
  REGION 1..125: note = Synthetic
QVQLVESGGGLEQPGGSLRLSCAGSGFTFRDYAMTWVRQAPGKGLEWVSSISGSGGNTYYADSVKGRFTISRDNSKNTLYLQMNSLRAEDTAVYYCAKDRLSITIRPRYYGLDVWGQGSTVTVSS

SEQ ID NO: 147 - DNA, 24 bp, synthetic construct
  misc_feature 1..24: note = Synthetic
  source 1..24: mol_type = other DNA
ggattcacctttagagactatgcc

SEQ ID NO: 148 - protein, 8 aa, synthetic construct
  REGION 1..8: note = Synthetic
GFTFRDYA

SEQ ID NO: 149 - DNA, 24 bp, synthetic construct
  misc_feature 1..24: note = Synthetic
  source 1..24: mol_type = other DNA
attagtggttccggtggtaacaca

SEQ ID NO: 150 - protein, 8 aa, synthetic construct
  REGION 1..8: note = Synthetic
ISGSGGNT

SEQ ID NO: 151 - DNA, 54 bp, synthetic construct; identical to SEQ ID NO: 55
  misc_feature 1..54: note = Synthetic
  source 1..54: mol_type = other DNA

SEQ ID NO: 152 - protein, 18 aa, synthetic construct
  REGION 1..18: note = Synthetic
AKDRLSITIRPRYYGLDV

SEQ ID NO: 153 - DNA, 339 bp, synthetic construct
  misc_feature 1..339: note = Synthetic
  source 1..339: mol_type = other DNA
gacatcgtgttgacccagtctccactctccctgcccgtcacccctggagagccggcctccatctcctgcaggtctagtcagagcctcctgtatagtattggatacaactatttggattggtacctgcagaagtcagggcagtctccacagctccttatctatttgggttctaatcgggcctccggggtccctgacaggttcagtggcagtggatcaggcacagattttacactgaaaatcagcagagtggaggctgaggatgttgggttttattactgcatgcaagctctacaaactccgtacacttttggccaggggaccaagctggagatcaaacga

SEQ ID NO: 154 - protein, 113 aa, synthetic construct
  REGION 1..113: note = Synthetic
DIVLTQSPLSLPVTPGEPASISCRSSQSLLYSIGYNYLDWYLQKSGQSPQLLIYLGSNRASGVPDRFSGSGSGTDFTLKISRVEAEDVGFYYCMQALQTPYTFGQGTKLEIKR

SEQ ID NO: 155 - DNA, 33 bp, synthetic construct; identical to SEQ ID NO: 83
  misc_feature 1..33: note = Synthetic
  source 1..33: mol_type = other DNA

SEQ ID NO: 156 - protein, 11 aa, synthetic construct
  REGION 1..11: note = Synthetic
QSLLYSIGYNY

SEQ ID NO: 157-158 - skipped (2 entries)

SEQ ID NO: 159 - DNA, 27 bp, synthetic construct
  misc_feature 1..27: note = Synthetic
  source 1..27: mol_type = other DNA
atgcaagctctacaaactccgtacact

SEQ ID NO: 160 - protein, 9 aa, synthetic construct
  REGION 1..9: note = Synthetic
MQALQTPYT

SEQ ID NO: 161 - DNA, 372 bp, synthetic construct
  misc_feature 1..372: note = Synthetic
  source 1..372: mol_type = other DNA
gaggtgcagctggtggagtctgggggaggcttggaacagccgggggggtccctgagactctcctgtgcaggctctggattcacctttagagactatgccatgacctgggtccgccaggctccagggaagggactggagtgggtctcatctattagtggttccggtggtaacacatactacgcagactccgtgaagggccggttcaccatctccagagacaattccaagaacacgctgtatctgcaaatgaacagcctgagagccgaggacacggccgtatattactgtgcgaaagatcgactctctataacaattcgcccacgctattatggtttggacgtctggggccaagggaccacggtcaccgtctcc

SEQ ID NO: 162 - protein, 124 aa, synthetic construct
  REGION 1..124: note = Synthetic
EVQLVESGGGLEQPGGSLRLSCAGSGFTFRDYAMTWVRQAPGKGLEWVSSISGSGGNTYYADSVKGRFTISRDNSKNTLYLQMNSLRAEDTAVYYCAKDRLSITIRPRYYGLDVWGQGTTVTVS

SEQ ID NO: 163 - DNA, 336 bp, synthetic construct
  misc_feature 1..336: note = Synthetic
  source 1..336: mol_type = other DNA
gacatcgtgatgacccagtctccactctccctgcccgtcacccctggagagccggcctccatctcctgcaggtctagtcagagcctcctgtatagtattggatacaactatttggattggtacctgcagaagtcagggcagtctccacagctccttatctatttgggttctaatcgggcctccggggtccctgacaggttcagtggcagtggatcaggcacagattttacactgaaaatcagcagagtggaggctgaggatgttgggttttattactgcatgcaagctctacaaactccgtacacttttggccaggggaccaagctggagatcaaa

SEQ ID NO: 164 - protein, 112 aa, synthetic construct [sequence omitted]

SEQ ID NO: 165 - DNA, 373 bp, synthetic construct
  misc_feature 1..373: note = Synthetic
  source 1..373: mol_type = other DNA
gaggtgcagctggtggagtctgggggaggcttggtacagcctggggggtccctgagactctcctgtgcagcctctggattcacctttagagactatgccatgagctgggtccgccaggctccagggaaggggctggagtgggtctcagctattagtggttccggtggtaacacatactacgcagactccgtgaagggccggttcaccatctccagagacaattccaagaacacgctgtatctgcaaatgaacagcctgagagccgaggacacggccgtatattactgtgcgaaagatcgactctctataacaattcgcccacgctattatggtttggacgtctggggccaagggaccacggtcaccgtctcct

SEQ ID NO: 166 - protein, 124 aa, synthetic construct; identical to SEQ ID NO: 70
  REGION 1..124: note = Synthetic

SEQ ID NO: 167 - DNA, 337 bp, synthetic construct; identical to SEQ ID NO: 95
  misc_feature 1..337: note = Synthetic
  source 1..337: mol_type = other DNA

SEQ ID NO: 168 - protein, 112 aa, synthetic construct; identical to SEQ ID NO: 96
  REGION 1..112: note = Synthetic

SEQ ID NO: 169 - DNA, 375 bp, synthetic construct
  misc_feature 1..375: note = Synthetic
  source 1..375: mol_type = other DNA
caggtgcagctggtggagtctgggggagtcttggagcagcctggggggtccctgagactctcctgtacagcctctggattcacctttagagactatgccatgacctgggtccgccaggctccagggaaggggctggagtgggtctcatctattagtggtagtggtggtaatacatactacgcagactccgtgaggggccggttcaccatctccagagacaactccaaccacacgctgtatctgcaaatgaacagcctgagagccgaagacacggccgtatattactgtgcgaaagatcgactctccataacaattcgcccacgctattacggtttggacgtctggggccaagggtccacggtcaccgtctcctca

SEQ ID NO: 170 - protein, 125 aa, synthetic construct
  REGION 1..125: note = Synthetic
QVQLVESGGVLEQPGGSLRLSCTASGFTFRDYAMTWVRQAPGKGLEWVSSISGSGGNTYYADSVRGRFTISRDNSNHTLYLQMNSLRAEDTAVYYCAKDRLSITIRPRYYGLDVWGQGSTVTVSS

SEQ ID NO: 171 - DNA, 24 bp, synthetic construct
  misc_feature 1..24: note = Synthetic
  source 1..24: mol_type = other DNA
ggattcacctttagagactatgcc

SEQ ID NO: 172 - protein, 8 aa, synthetic construct
  REGION 1..8: note = Synthetic
GFTFRDYA

SEQ ID NO: 173 - DNA, 24 bp, synthetic construct
  misc_feature 1..24: note = Synthetic
  source 1..24: mol_type = other DNA
attagtggtagtggtggtaataca

SEQ ID NO: 174 - protein, 8 aa, synthetic construct
  REGION 1..8: note = Synthetic
ISGSGGNT

SEQ ID NO: 175 - DNA, 54 bp, synthetic construct
  misc_feature 1..54: note = Synthetic
  source 1..54: mol_type = other DNA
gcgaaagatcgactctccataacaattcgcccacgctattacggtttggacgtc

SEQ ID NO: 176 - protein, 18 aa, synthetic construct
  REGION 1..18: note = Synthetic
AKDRLSITIRPRYYGLDV

SEQ ID NO: 177 - DNA, 324 bp, synthetic construct
  misc_feature 1..324: note = Synthetic
  source 1..324: mol_type = other DNA
gatattgtgatgacccagtctccatcctccctgtctgcatctgtaggagacagagtcaccattacttgccgggcgagtcaggacattagcaattattttgcctggtatcagcagaagccagggaaagttcctaaactcctgatctttgctgcatccactttgcatccaggggtcccatctcggttcagtggcagtggatctgggacagatttcactctcaccattagtagcctgcagcctgaagatgttgcaacttattactgtcaaaagtataacagtgccccgtacacttttggccaggggaccaaggtggaaatcaaacga

SEQ ID NO: 178 - protein, 108 aa, synthetic construct
  REGION 1..108: note = Synthetic
DIVMTQSPSSLSASVGDRVTITCRASQDISNYFAWYQQKPGKVPKLLIFAASTLHPGVPSRFSGSGSGTDFTLTISSLQPEDVATYYCQKYNSAPYTFGQGTKVEIKR

SEQ ID NO: 179 - DNA, 18 bp, synthetic construct
  misc_feature 1..18: note = Synthetic
  source 1..18: mol_type = other DNA
caggacattagcaattat

SEQ ID NO: 180 - protein, 6 aa, synthetic construct
  REGION 1..6: note = Synthetic
QDISNY

SEQ ID NO: 181-182 - skipped (2 entries)

SEQ ID NO: 183 - DNA, 27 bp, synthetic construct
  misc_feature 1..27: note = Synthetic
  source 1..27: mol_type = other DNA
caaaagtataacagtgccccgtacact

SEQ ID NO: 184 - protein, 9 aa, synthetic construct
  REGION 1..9: note = Synthetic
QKYNSAPYT

SEQ ID NO: 185 - DNA, 372 bp, synthetic construct
  misc_feature 1..372: note = Synthetic
  source 1..372: mol_type = other DNA
gaggtgcagctggtggagtctgggggagtcttggagcagcctggggggtccctgagactctcctgtacagcctctggattcacctttagagactatgccatgacctgggtccgccaggctccagggaaggggctggagtgggtctcatctattagtggtagtggtggtaatacatactacgcagactccgtgaggggccggttcaccatctccagagacaactccaaccacacgctgtatctgcaaatgaacagcctgagagccgaagacacggccgtatattactgtgcgaaagatcgactctccataacaattcgcccacgctattacggtttggacgtctggggccaagggaccacggtcaccgtctcc

SEQ ID NO: 186 - protein, 124 aa, synthetic construct
  REGION 1..124: note = Synthetic
EVQLVESGGVLEQPGGSLRLSCTASGFTFRDYAMTWVRQAPGKGLEWVSSISGSGGNTYYADSVRGRFTISRDNSNHTLYLQMNSLRAEDTAVYYCAKDRLSITIRPRYYGLDVWGQGTTVTVS

SEQ ID NO: 187 - DNA, 321 bp, synthetic construct
  misc_feature 1..321: note = Synthetic
  source 1..321: mol_type = other DNA
gacatccagatgacccagtctccatcctccctgtctgcatctgtaggagacagagtcaccattacttgccgggcgagtcaggacattagcaattattttgcctggtatcagcagaagccagggaaagttcctaaactcctgatctttgctgcatccactttgcatccaggggtcccatctcggttcagtggcagtggatctgggacagatttcactctcaccattagtagcctgcagcctgaagatgttgcaacttattactgtcaaaagtataacagtgccccgtacacttttggccaggggaccaagctggagatcaaa

SEQ ID NO: 188 - protein, 107 aa, synthetic construct
  REGION 1..107: note = Synthetic
DIQMTQSPSSLSASVGDRVTITCRASQDISNYFAWYQQKPGKVPKLLIFAASTLHPGVPSRFSGSGSGTDFTLTISSLQPEDVATYYCQKYNSAPYTFGQGTKLEIK

SEQ ID NO: 189 - DNA, 373 bp, synthetic construct
  misc_feature 1..373: note = Synthetic
  source 1..373: mol_type = other DNA
gaggtgcagctggtggagtctgggggaggcttggtacagcctggggggtccctgagactctcctgtgcagcctctggattcacctttagagactatgccatgagctgggtccgccaggctccagggaaggggctggagtgggtctcagctattagtggtagtggtggtaatacatactacgcagactccgtgaagggccggttcaccatctccagagacaattccaagaacacgctgtatctgcaaatgaacagcctgagagccgaggacacggccgtatattactgtgcgaaagatcgactctccataacaattcgcccacgctattacggtttggacgtctggggccaagggaccacggtcaccgtctcct

SEQ ID NO: 190 - protein, 124 aa, synthetic construct; identical to SEQ ID NO: 70
  REGION 1..124: note = Synthetic

SEQ ID NO: 191 - DNA, 322 bp, synthetic construct
  misc_feature 1..322: note = Synthetic
  source 1..322: mol_type = other DNA
gacatccagatgacccagtctccatcctccctgtctgcatctgtaggagacagagtcaccatcacttgccgggcgagtcaggacattagcaattatttagcctggtatcagcagaaaccagggaaagttcctaagctcctgatctatgctgcatccactttgcaatcaggggtcccatctcggttcagtggcagtggatctgggacagatttcactctcaccatcagcagcctgcagcctgaagatgttgcaacttattactgtcaaaagtataacagtgccccgtacacttttggccaggggaccaagctggagatcaaac

SEQ ID NO: 192 - protein, 107 aa, synthetic construct
  REGION 1..107: note = Synthetic
DIQMTQSPSSLSASVGDRVTITCRASQDISNYLAWYQQKPGKVPKLLIYAASTLQSGVPSRFSGSGSGTDFTLTISSLQPEDVATYYCQKYNSAPYTFGQGTKLEIK

SEQ ID NO: 193 - DNA, 355 bp, synthetic construct
  misc_feature 1..355: note = Synthetic
  source 1..355: mol_type = other DNA
gaagtgcacctggtggaatctgggggaggcttggtacagcctggcaggtccctgagactctcctgtgaggcctctggattcacctttgatgattatgccatgcactgggtccggcaagctccggggaagggcctggaatgggtctcaggtcttagtcggacaagtgtcagtataggctatgcggactctgtgaagggccgattcaccatctccagagacaacgccaagaactccctttatttggaaatgaacagtctgagacctgaggacacggccttatattactgtgcaaaatgggggacccgggggtattttgactactggggccagggaaccctggtcaccgtctcctcag

SEQ ID NO: 194 - protein, 118 aa, synthetic construct
  REGION 1..118: note = Synthetic
EVHLVESGGGLVQPGRSLRLSCEASGFTFDDYAMHWVRQAPGKGLEWVSGLSRTSVSIGYADSVKGRFTISRDNAKNSLYLEMNSLRPEDTALYYCAKWGTRGYFDYWGQGTLVTVSS

SEQ ID NO: 195 - DNA, 24 bp, synthetic construct
  misc_feature 1..24: note = Synthetic
  source 1..24: mol_type = other DNA
ggattcacctttgatgattatgcc

SEQ ID NO: 196 - protein, 8 aa, synthetic construct
  REGION 1..8: note = Synthetic
GFTFDDYA

SEQ ID NO: 197 - DNA, 24 bp, synthetic construct
  misc_feature 1..24: note = Synthetic
  source 1..24: mol_type = other DNA
cttagtcggacaagtgtcagtata

SEQ ID NO: 198 - protein, 8 aa, synthetic construct
  REGION 1..8: note = Synthetic
LSRTSVSI

SEQ ID NO: 199 - DNA, 33 bp, synthetic construct
  misc_feature 1..33: note = Synthetic
  source 1..33: mol_type = other DNA
gcaaaatgggggacccgggggtattttgactac

SEQ ID NO: 200 - protein, 11 aa, synthetic construct
  REGION 1..11: note = Synthetic
AKWGTRGYFDY

SEQ ID NO: 201 - DNA, 322 bp, synthetic construct
  misc_feature 1..322: note = Synthetic
  source 1..322: mol_type = other DNA
gacatccagatgacccagtctccatcttccgtgtctgcatctgtgggagacagagtcaccatcacttgtcgggcgagtcaggatattagtatttggttagcctggtatcagcagagtccagggaaagcccctaaactcctgatcaatgttgcatcccgtttgcaaagtggggtcccatcaaggttcagcggcagtggatctgggacagatttcactctcaccatcaacagtctgcagcctgaagattttgtaacttactattgtcaacaggctaacagtttcccgatcaccttcggccaagggacacgactggcgaccaaac

SEQ ID NO: 202 - protein, 107 aa, synthetic construct
  REGION 1..107: note = Synthetic
DIQMTQSPSSVSASVGDRVTITCRASQDISIWLAWYQQSPGKAPKLLINVASRLQSGVPSRFSGSGSGTDFTLTINSLQPEDFVTYYCQQANSFPITFGQGTRLATK

SEQ ID NO: 203 - DNA, 18 bp, synthetic construct
  misc_feature 1..18: note = Synthetic
  source 1..18: mol_type = other DNA
caggatattagtatttgg

SEQ ID NO: 204 - protein, 6 aa, synthetic construct
  REGION 1..6: note = Synthetic
QDISIW

SEQ ID NO: 205-206 - skipped (2 entries)

SEQ ID NO: 207 - DNA, 27 bp, synthetic construct
  misc_feature 1..27: note = Synthetic
  source 1..27: mol_type = other DNA
caacaggctaacagtttcccgatcacc

SEQ ID NO: 208 - protein, 9 aa, synthetic construct
  REGION 1..9: note = Synthetic
QQANSFPIT

SEQ ID NO: 209 - DNA, 355 bp, synthetic construct
  misc_feature 1..355: note = Synthetic
  source 1..355: mol_type = other DNA
gaggtgcagctggtggagtctgggggaggcttggtacagcctggcaggtccctgagactctcctgtgaggcctctggattcacctttgatgattatgccatgcactgggtccggcaagctccggggaagggcctggaatgggtctcaggtcttagtcggacaagtgtcagtataggctatgcggactctgtgaagggccgattcaccatctccagagacaacgccaagaactccctttatttggaaatgaacagtctgagacctgaggacacggccttatattactgtgcaaaatgggggacccgggggtattttgactactggggccagggaaccctggtcaccgtctcctcag

SEQ ID NO: 210 - protein, 118 aa, synthetic construct
  REGION 1..118: note = Synthetic
EVQLVESGGGLVQPGRSLRLSCEASGFTFDDYAMHWVRQAPGKGLEWVSGLSRTSVSIGYADSVKGRFTISRDNAKNSLYLEMNSLRPEDTALYYCAKWGTRGYFDYWGQGTLVTVSS

SEQ ID NO: 211 - DNA, 322 bp, synthetic construct
  misc_feature 1..322: note = Synthetic
  source 1..322: mol_type = other DNA
gacatccagatgacccagtctccatcttccgtgtctgcatctgtgggagacagagtcaccatcacttgtcgggcgagtcaggatattagtatttggttagcctggtatcagcagagtccagggaaagcccctaaactcctgatcaatgttgcatcccgtttgcaaagtggggtcccatcaaggttcagcggcagtggatctgggacagatttcactctcaccatcaacagtctgcagcctgaagattttgtaacttactattgtcaacaggctaacagtttcccgatcaccttcggccaagggacacgactggagattaaac

SEQ ID NO: 212 - protein, 107 aa, synthetic construct
  REGION 1..107: note = Synthetic
DIQMTQSPSSVSASVGDRVTITCRASQDISIWLAWYQQSPGKAPKLLINVASRLQSGVPSRFSGSGSGTDFTLTINSLQPEDFVTYYCQQANSFPITFGQGTRLEIK

SEQ ID NO: 213 - DNA, 355 bp, synthetic construct
  misc_feature 1..355: note = Synthetic
  source 1..355: mol_type = other DNA
gaagtgcagctggtggagtctgggggaggcttggtacagcctggcaggtccctgagactctcctgtgcagcctctggattcacctttgatgattatgccatgcactgggtccggcaagctccagggaagggcctggagtgggtctcaggtcttagtcggacaagtgtcagtataggctatgcggactctgtgaagggccgattcaccatctccagagacaacgccaagaactccctgtatctgcaaatgaacagtctgagagctgaggacacggccttgtattactgtgcaaaatgggggacccgggggtattttgactactggggccaaggaaccctggtcaccgtctcctcag

SEQ ID NO: 214 - protein, 118 aa, synthetic construct
  REGION 1..118: note = Synthetic
EVQLVESGGGLVQPGRSLRLSCAASGFTFDDYAMHWVRQAPGKGLEWVSGLSRTSVSIGYADSVKGRFTISRDNAKNSLYLQMNSLRAEDTALYYCAKWGTRGYFDYWGQGTLVTVSS

SEQ ID NO: 215 - DNA, 322 bp, synthetic construct
  misc_feature 1..322: note = Synthetic
  source 1..322: mol_type = other DNA
gacatccagatgacccagtctccatcttccgtgtctgcatctgtaggagacagagtcaccatcacttgtcgggcgagtcaggatattagtatttggttagcctggtatcagcagaaaccagggaaagcccctaagctcctgatctatgttgcatccagtttgcaaagtggggtcccatcaaggttcagcggcagtggatctgggacagatttcactctcaccatcagcagcctgcagcctgaagattttgcaacttactattgtcaacaggctaacagtttcccgatcaccttcggccaagggacacgactggagattaaac

SEQ ID NO: 216 - protein, 107 aa, synthetic construct
  REGION 1..107: note = Synthetic
DIQMTQSPSSVSASVGDRVTITCRASQDISIWLAWYQQKPGKAPKLLIYVASSLQSGVPSRFSGSGSGTDFTLTISSLQPEDFATYYCQQANSFPITFGQGTRLEIK

SEQ ID NO: 217 - DNA, 363 bp, synthetic construct
  misc_feature 1..363: note = Synthetic
  source 1..363: mol_type = other DNA
gaggtgcagctgttggagtctgggggaggcttgctacagccgggggggtccctgagactctcctgtgcagcctctggaatcacctttagcacctatgccatgagctgggtccgtcaggctccagggagggggctggagtgggtctcagctattagtggtagtggtgatagcacatcctacgcagactccgtgaagggccggttcaccagctccagagacaattccaagaacacgctgtatctgcaaatgaacagcctgagagccgaggacacggccgtatattactgtgcgaaagtcatagcagctcgtcctcactggaacttcgatctctggggccgtggcaccctggtcactgtctcctca

SEQ ID NO: 218 - protein, 121 aa, synthetic construct
  REGION 1..121: note = Synthetic
EVQLLESGGGLLQPGGSLRLSCAASGITFSTYAMSWVRQAPGRGLEWVSAISGSGDSTSYADSVKGRFTSSRDNSKNTLYLQMNSLRAEDTAVYYCAKVIAARPHWNFDLWGRGTLVTVSS

SEQ ID NO: 219 - DNA, 24 bp, synthetic construct
  misc_feature 1..24: note = Synthetic
  source 1..24: mol_type = other DNA
ggaatcacctttagcacctatgcc

SEQ ID NO: 220 - protein, 8 aa, synthetic construct
  REGION 1..8: note = Synthetic
GITFSTYA

SEQ ID NO: 221 - DNA, 24 bp, synthetic construct
  misc_feature 1..24: note = Synthetic
  source 1..24: mol_type = other DNA
attagtggtagtggtgatagcaca

SEQ ID NO: 222 - protein, 8 aa, synthetic construct
  REGION 1..8: note = Synthetic
ISGSGDST

SEQ ID NO: 223 - DNA, 42 bp, synthetic construct
  misc_feature 1..42: note = Synthetic
  source 1..42: mol_type = other DNA
gcgaaagtcatagcagctcgtcctcactggaacttcgatctc

SEQ ID NO: 224 - protein, 14 aa, synthetic construct
  REGION 1..14: note = Synthetic
AKVIAARPHWNFDL

SEQ ID NO: 225 - DNA, 324 bp, synthetic construct
  misc_feature 1..324: note = Synthetic
  source 1..324: mol_type = other DNA
gaaattgtgttgacacagtctccagccaccctgtctttgtctccaggggaaagagccaccctctcctgcagggccagtcagagtgttagtagatatttagcctggtatcaacagaaacctggccaggctcccaggctcctcatctatgatgcatccaacagggccactggcatcccagccaggttcagtggcagtgggtctgggacagacttcactctcaccatcagcagcctagagcctgaagattttggagtttattactgtcagcagcgtagtgactggccgctcactttcggcggagggaccaaggtggagatcaaacgg

SEQ ID NO: 226 - protein, 107 aa, synthetic construct
  REGION 1..107: note = Synthetic
EIVLTQSPATLSLSPGERATLSCRASQSVSRYLAWYQQKPGQAPRLLIYDASNRATGIPARFSGSGSGTDFTLTISSLEPEDFGVYYCQQRSDWPLTFGGGTKVEIK

SEQ ID NO: 227 - DNA, 18 bp, synthetic construct
  misc_feature 1..18: note = Synthetic
  source 1..18: mol_type = other DNA
cagagtgttagtagatat

SEQ ID NO: 228 - protein, 6 aa, synthetic construct
  REGION 1..6: note = Synthetic
QSVSRY

SEQ ID NO: 229-230 - skipped (2 entries)

SEQ ID NO: 231 - DNA, 27 bp, synthetic construct
  misc_feature 1..27: note = Synthetic
  source 1..27: mol_type = other DNA
cagcagcgtagtgactggccgctcact

SEQ ID NO: 232 - protein, 9 aa, synthetic construct
  REGION 1..9: note = Synthetic
QQRSDWPLT

SEQ ID NO: 233 - DNA, 363 bp, synthetic construct; identical to SEQ ID NO: 217
  misc_feature 1..363: note = Synthetic
  source 1..363: mol_type = other DNA

SEQ ID NO: 234 - protein, 121 aa, synthetic construct; identical to SEQ ID NO: 218
  REGION 1..121: note = Synthetic

SEQ ID NO: 235 - DNA, 324 bp, synthetic construct; identical to SEQ ID NO: 225
  misc_feature 1..324: note = Synthetic
  source 1..324: mol_type = other DNA

SEQ ID NO: 236 - protein, 107 aa, synthetic construct; identical to SEQ ID NO: 226
  REGION 1..107: note = Synthetic

SEQ ID NO: 237 - DNA, 363 bp, synthetic construct
  misc_feature 1..363: note = Synthetic
  source 1..363: mol_type = other DNA
gaggtgcagctgttggagtctgggggaggcttggtacagccgggggggtccctgagactctcctgtgcagcctctggaatcacctttagcacctatgccatgagctgggtccgtcaggctccagggaaggggctggagtgggtctcagctattagtggtagtggtgatagcacatactacgcagactccgtgaagggccggttcaccatctccagagacaattccaagaacacgctgtatctgcaaatgaacagcctgagagccgaggacacggccgtatattactgtgcgaaagtcatagcagctcgtcctcactggaacttcgatctctggggccgtggcaccctggtcactgtctcctca

SEQ ID NO: 238 - protein, 121 aa, synthetic construct
  REGION 1..121: note = Synthetic
EVQLLESGGGLVQPGGSLRLSCAASGITFSTYAMSWVRQAPGKGLEWVSAISGSGDSTYYADSVKGRFTISRDNSKNTLYLQMNSLRAEDTAVYYCAKVIAARPHWNFDLWGRGTLVTVSS

SEQ ID NO: 239 - DNA, 324 bp, synthetic construct
  misc_feature 1..324: note = Synthetic
  source 1..324: mol_type = other DNA
gaaattgtgttgacacagtctccagccaccctgtctttgtctccaggggaaagagccaccctctcctgcagggccagtcagagtgttagtagatatttagcctggtatcaacagaaacctggccaggctcccaggctcctcatctatgatgcatccaacagggccactggcatcccagccaggttcagtggcagtgggtctgggacagacttcactctcaccatcagcagcctagagcctgaagattttgcagtttattactgtcagcagcgtagtgactggccgctcactttcggcggagggaccaaggtggagatcaaacgg

SEQ ID NO: 240 - protein, 108 aa, synthetic construct
  REGION 1..108: note = Synthetic
EIVLTQSPATLSLSPGERATLSCRASQSVSRYLAWYQQKPGQAPRLLIYDASNRATGIPARFSGSGSGTDFTLTISSLEPEDFAVYYCQQRSDWPLTFGGGTKVEIKR

SEQ ID NO: 241 - DNA, 366 bp, synthetic construct
  misc_feature 1..366: note = Synthetic
  source 1..366: mol_type = other DNA
caggtgcagctggtggagtctgggggaggcgtggtccagcctgggaggtccctgagactcacctgtgcagcctctggattcaccttcagtagtaatggcatgcactgggtccgccaggctccaggcaaggggctggagtgggtggcaattatatcatatgatggaaataatcaatactatgcagactccgtgaagggccgattcaccatctccagagacaattccaagcacacgctgtatctggaaatgaacagcctgagagctgaggacacggctgtgtattactgtacaaaagccatctctataagtggaacttacaactggttcgattcctggggccagggaaccctggtcaccgtctcctca

SEQ ID NO: 242 - protein, 122 aa, synthetic construct
  REGION 1..122: note = Synthetic
QVQLVESGGGVVQPGRSLRLTCAASGFTFSSNGMHWVRQAPGKGLEWVAIISYDGNNQYYADSVKGRFTISRDNSKHTLYLEMNSLRAEDTAVYYCTKAISISGTYNWFDSWGQGTLVTVSS

SEQ ID NO: 243 - DNA, 24 bp, synthetic construct
  misc_feature 1..24: note = Synthetic
  source 1..24: mol_type = other DNA
ggattcaccttcagtagtaatggc

SEQ ID NO: 244 - protein, 8 aa, synthetic construct
  REGION 1..8: note = Synthetic
GFTFSSNG

SEQ ID NO: 245 - DNA, 24 bp, synthetic construct
  misc_feature 1..24: note = Synthetic
  source 1..24: mol_type = other DNA
atatcatatgatggaaataatcaa

SEQ ID NO: 246 - protein, 8 aa, synthetic construct
  REGION 1..8: note = Synthetic
ISYDGNNQ

SEQ ID NO: 247 - DNA, 45 bp, synthetic construct
  misc_feature 1..45: note = Synthetic
  source 1..45: mol_type = other DNA
acaaaagccatctctataagtggaacttacaactggttcgattcc

SEQ ID NO: 248 - protein, 15 aa, synthetic construct
  REGION 1..15: note = Synthetic
TKAISISGTYNWFDS

SEQ ID NO: 249 - DNA, 324 bp, synthetic construct
  misc_feature 1..324: note = Synthetic
  source 1..324: mol_type = other DNA
gaaattgtattgacacagtctccagccatcctgtctttgtctccaggggaaagagccaccctctcctgcagggccagtcagagtgttagcaggtacttagcctggtaccaacagaaacctggccaggctcccaggctcctcatctatgatgcatccaacagggccactggcatcccagccaggttcagtggcagtgggtctgggacagacttcactctcaccatcagcagcctagagcctgaagattttgcagtttattactgtcaacagcgtagcaactggccgctcactttcggcggagggaccaaggtggagatcaaacgg

SEQ ID NO: 250 - protein, 107 aa, synthetic construct
  REGION 1..107: note = Synthetic
EIVLTQSPAILSLSPGERATLSCRASQSVSRYLAWYQQKPGQAPRLLIYDASNRATGIPARFSGSGSGTDFTLTISSLEPEDFAVYYCQQRSNWPLTFGGGTKVEIK

SEQ ID NO: 251 - DNA, 18 bp, synthetic construct
  misc_feature 1..18: note = Synthetic
  source 1..18: mol_type = other DNA
cagagtgttagcaggtac

SEQ ID NO: 252 - protein, 6 aa, synthetic construct
  REGION 1..6: note = Synthetic
QSVSRY

SEQ ID NO: 253-254 - skipped (2 entries)

SEQ ID NO: 255 - DNA, 27 bp, synthetic construct
  misc_feature 1..27: note = Synthetic
  source 1..27: mol_type = other DNA
caacagcgtagcaactggccgctcact

SEQ ID NO: 256 - protein, 9 aa, synthetic construct
  REGION 1..9: note = Synthetic
QQRSNWPLT

SEQ ID NO: 257 - DNA, 366 bp, synthetic construct; identical to SEQ ID NO: 241
  misc_feature 1..366: note = Synthetic
  source 1..366: mol_type = other DNA

SEQ ID NO: 258 - protein, 122 aa, synthetic construct; identical to SEQ ID NO: 242
  REGION 1..122: note = Synthetic

SEQ ID NO: 259 - DNA, 324 bp, synthetic construct; identical to SEQ ID NO: 249
  misc_feature 1..324: note = Synthetic
  source 1..324: mol_type = other DNA

SEQ ID NO: 260 - protein, 107 aa, synthetic construct; identical to SEQ ID NO: 250
  REGION 1..107: note = Synthetic

SEQ ID NO: 261 - DNA, 366 bp, synthetic construct
  misc_feature 1..366: note = Synthetic
  source 1..366: mol_type = other DNA
caggtgcagctggtggagtctgggggaggcgtggtccagcctgggaggtccctgagactctcctgtgcagcctctggattcaccttcagtagtaatggcatgcactgggtccgccaggctccaggcaaggggctggagtgggtggcagttatatcatatgatggaaataatcaatactatgcagactccgtgaagggccgattcaccatctccagagacaattccaagaacacgctgtatctgcaaatgaacagcctgagagctgaggacacggctgtgtattactgtacaaaagccatctctataagtggaacttacaactggttcgattcctggggccagggaaccctggtcaccgtctcctca

SEQ ID NO: 262 - protein, 122 aa, synthetic construct
  REGION 1..122: note = Synthetic
QVQLVESGGGVVQPGRSLRLSCAASGFTFSSNGMHWVRQAPGKGLEWVAVISYDGNNQYYADSVKGRFTISRDNSKNTLYLQMNSLRAEDTAVYYCTKAISISGTYNWFDSWGQGTLVTVSS

SEQ ID NO: 263 - DNA, 324 bp, synthetic construct
  misc_feature 1..324: note = Synthetic
  source 1..324: mol_type = other DNA
gaaattgtattgacacagtctccagccaccctgtctttgtctccaggggaaagagccaccctctcctgcagggccagtcagagtgttagcaggtacttagcctggtaccaacagaaacctggccaggctcccaggctcctcatctatgatgcatccaacagggccactggcatcccagccaggttcagtggcagtgggtctgggacagacttcactctcaccatcagcagcctagagcctgaagattttgcagtttattactgtcaacagcgtagcaactggccgctcactttcggcggagggaccaaggtggagatcaaacgg

SEQ ID NO: 264 - protein, 108 aa, synthetic construct
  REGION 1..108: note = Synthetic
EIVLTQSPATLSLSPGERATLSCRASQSVSRYLAWYQQKPGQAPRLLIYDASNRATGIPARFSGSGSGTDFTLTISSLEPEDFAVYYCQQRSNWPLTFGGGTKVEIKR

SEQ ID NO: 265-270 - skipped (6 entries)

SEQ ID NO: 271 - protein, 330 aa, synthetic construct [sequence omitted]

SEQ ID NO: 272 - protein, 327 aa, synthetic construct
  REGION 1..327: note = Synthetic
ASTKGPSVFPLAPCSRSTSESTAALGCLVKDYFPEPVTVSWNSGALTSGVHTFPAVLQSSGLYSLSSVVTVPSSSLGTKTYTCNVDHKPSNTKVDKRVESKYGPPCPSCPAPEFLGGPSVFLFPPKPKDTLMISRTPEVTCVVVDVSQEDPEVQFNWYVDGVEVHNAKTKPREEQFNSTYRVVSVLTVLHQDWLNGKEYKCKVSNKGLPSSIEKTISKAKGQPREPQVYTLPPSQEEMTKNQVSLTCLVKGFYPSDIAVEWESNGQPENNYKTTPPVLDSDGSFFLYSRLTVDKSRWQEGNVFSCSVMHEALHNHYTQKSLSLSLGK

SEQ ID NO: 273 - protein, 327 aa, synthetic construct
  REGION 1..327: note = Synthetic
ASTKGPSVFPLAPCSRSTSESTAALGCLVKDYFPEPVTVSWNSGALTSGVHTFPAVLQSSGLYSLSSVVTVPSSSLGTKTYTCNVDHKPSNTKVDKRVESKYGPPCPPCPAPEFLGGPSVFLFPPKPKDTLMISRTPEVTCVVVDVSQEDPEVQFNWYVDGVEVHNAKTKPREEQFNSTYRVVSVLTVLHQDWLNGKEYKCKVSNKGLPSSIEKTISKAKGQPREPQVYTLPPSQEEMTKNQVSLTCLVKGFYPSDIAVEWESNGQPENNYKTTPPVLDSDGSFFLYSRLTVDKSRWQEGNVFSCSVMHEALHNHYTQKSLSLSLGK

SEQ ID NO: 274 - protein, 207 aa, Homo sapiens
MKVLQEPTCVSDYMSISTCEWKMNGPTNCSTELRLLYQLVFLLSEAHTCIPENNGGAGCVCHLLMDDVVSADNYTLDLWAGQQLLWKGSFKPSEHVKPRAPGNLTVHTNVSDTLLLTWSNPYPPDNYLYNHLTYAVNIWSENDPADFRIYNVTYLEPSLRIAASTLKSGISYRARVRAWAQCYNTTWSEWSPSTKWHNSYREPFEQH

SEQ ID NO: 275 - protein, 231 aa, Macaca fascicularis
MGWLCSGLLFPVSCLVLLQVASSGSMKVLQEPTCVSDYMSISTCEWKMGGPTNCSAELRLLYQLVFQSSETHTCVPENNGGVGCVCHLLMDDVVSMDNYTLDLWAGQQLLWKGSFKPSEHVKPRAPGNLTVHTNVSDTVLLTWSNPYPPDNYLYNDLTYAVNIWSENDPAYSRIHNVTYLKPTLRIPASTLKSGISYRARVRAWAQHYNTTWSEWSPSTKWYNSYREPFEQ